European Patent Specification EP 3 807 635 B1, published April 9, 2025. Title: Méthode de Stratification du Risque de Néphropathie à BK-virus après Transplantation Rénale. Applicant: INSTITUT NATIONAL DE LA SANTE ET DE LA RECHERCHE MEDICALE (INSERM) ASSISTANCE PUBLIQUE - HOPITAUX DE PARIS UNIVERSITE PARIS-SUD. The sequence listing filed with the application follows.

SEQUENCE LISTING (3 sequences)

SEQ ID NO: 1 - DNA, 20 bp, ARTIFICIAL
  amorce sens de 5'-3' pour amplifier BK-V
catagcatgcaagggcagtg

SEQ ID NO: 2 - DNA, 20 bp, artificial
  Amorce antisens de 5' en 3' pour amplifier BK-V
gagctgcctggggaaatctt

SEQ ID NO: 3 - DNA, 20 bp, artificial
  sonde PCR
taggccattccttgcagtac